European Patent Application EP 4 779 024 A2, published July 22, 2026. Title: Modified AAV capsid polypeptides for Treatment of Muscular Diseases. Applicant: Universität Heidelberg. Application EP. The sequence listing filed with the application follows.

SEQUENCE LISTING (55 sequences)

SEQ ID NO: 1 - skipped

SEQ ID NO: 2 - protein, 7 aa, synthetic construct
  REGION 1..7: note = binding peptide P1
RGDLGLS

SEQ ID NO: 3 - protein, 7 aa, synthetic construct
  REGION 1..7: note = binding paptide P3
RGDAVGV

SEQ ID NO: 4 - protein, 8 aa, synthetic construct
  REGION 1..8: note = binding peptide A1
MPLGAAGA

SEQ ID NO: 5 - protein, 8 aa, synthetic construct
  REGION 1..8: note = binding peptide K3
RGDLRVSA

SEQ ID NO: 6 - protein, 7 aa, synthetic construct
  REGION 1..7: note = binding peptide MTP
ASSLNIA

SEQ ID NO: 7 - protein, 21 aa, synthetic construct
  REGION 1..21: note = AAV9_P1 insertion site
NHQGQSGRGDLGLSAQAAQTG

SEQ ID NO: 8 - protein, 21 aa, synthetic construct
  REGION 1..21: note = AAV9_P3 insertion site
NHQGQSGRGDAVGVAQAAQTG

SEQ ID NO: 9 - protein, 21 aa, synthetic construct
  REGION 1..21: note = AAVpo1_A1 insertion site
NNQGQRGMPLGAAGAQAATVG

SEQ ID NO: 10 - protein, 21 aa, synthetic construct
  REGION 1..21: note = AAV9_K3 insertion site
HQSGQAGRGDLRVSAQAATGW

SEQ ID NO: 11 - protein, 21 aa, synthetic construct
  REGION 1..21: note = AAV-MTP insertion site
NLQRGNTGASSLNIAGLSRQA

SEQ ID NO: 12 - protein, 770 aa, synthetic construct
  REGION 1..745: note = AAV9_P1 capsid polypeptide, insertion site 588
MAADGYLPDWLEDNLSEGIREWWALKPGAPQPKANQQHQDNARGLVLPGYKYLGPGNGLDKGEPVNAADAAALEHDKAYDQQLKAGDNPYLKYNHADAEFQERLKEDTSFGGNLGRAVFQAKKRLLEPLGLVEEAAKTAPGKKRPVEQSPQEPDSSAGIGKSGAQPAKKRLNFGQTGDTESVPDPQPIGEPPAAPSGVGSLTMASGGGAPVADNNEGADGVGSSSGNWHCDSQWLGDRVITTSTRTWALPTYNNHLYKQISNSTSGGSSNDNAYFGYSTPWGYFDFNRFHCHFSPRDWQRLINNNWGFRPKRLNFKLFNIQVKEVTDNNGVKTIANNLTSTVQVFTDSDYQLPYVLGSAHEGCLPPFPADVFMIPQYGYLTLNDGSQAVGRSSFYCLEYFPSQMLRTGNNFQFSYEFENVPFHSSYAHSQSLDRLMNPLIDQYLYYLSKTINGSGQNQQTLKFSVAGPSNMAVQGRNYIPGPSYRQQRVSTTVTQNNNSEFAWPGASSWALNGRNSLMNPGPAMASHKEGEDRFFPLSGSLIFGKQGTGRDNVDADKVMITNEEEIKTTNPVATESYGQVATNHQGQSGRGDLGLSAQAAQTGWVQNQGILPGMVWQDRDVYLQGPIWAKIPHTDGNFHPSPLMGGFGMKHPPPQILIKNTPVPADPPTAFNKDKLNSFITQYSTGQVSVEIEWELQKENSKRWNPEIQYTSNYYKSNNVEFAVNTEGVYSEPRPIGTRYLTRNLEFAVNTEGVYSEPRPIGTRYLTRNL

SEQ ID NO: 13 - DNA, 2238 bp, synthetic construct
  misc_feature 1..2238: note = AAV9_P1 capsid polypeptide encoding, insertion site amino acid 588
  source 1..2238: mol_type = other DNA
atggctgccgatggttatcttccagattggctcgaggacaaccttagtgaaggaattcgcgagtggtgggctttgaaacctggagcccctcaacccaaggcaaatcaacaacatcaagacaacgctcgaggtcttgtgcttccgggttacaaataccttggacccggcaacggactcgacaagggggagccggtcaacgcagcagacgcggcggccctcgagcacgacaaggcctacgaccagcagctcaaggccggagacaacccgtacctcaagtacaaccacgccgacgccgagttccaggagcggctcaaagaagatacgtcttttgggggcaacctcgggcgagcagtcttccaggccaaaaagaggcttcttgaacctcttggtctggttgaggaagcggctaagacggctcctggaaagaagaggcctgtagagcagtctcctcaggaaccggactcctccgcgggtattggcaaatcgggtgcacagcccgctaaaaagagactcaatttcggtcagactggcgacacagagtcagtcccagaccctcaaccaatcggagaacctcccgcagccccctcaggtgtgggatctcttacaatggcttcaggtggtggcgcaccagtggcagacaataacgaaggtgccgatggagtgggtagttcctcgggaaattggcattgcgattcccaatggctgggggacagagtcatcaccaccagcacccgaacctgggccctgcccacctacaacaatcacctctacaagcaaatctccaacagcacatctggaggatcttcaaatgacaacgcctacttcggctacagcaccccctgggggtattttgacttcaacagattccactgccacttctcaccacgtgactggcagcgactcatcaacaacaactggggattccggcctaagcgactcaacttcaagctcttcaacattcaggtcaaagaggttacggacaacaatggagtcaagaccatcgccaataaccttaccagcacggtccaggtcttcacggactcagactatcagctcccgtacgtgctcgggtcggctcacgagggctgcctcccgccgttcccagcggacgttttcatgattcctcagtacgggtatctgacgcttaatgatggaagccaggccgtgggtcgttcgtccttttactgcctggaatatttcccgtcgcaaatgctaagaacgggtaacaacttccagttcagctacgagtttgagaacgtacctttccatagcagctacgctcacagccaaagcctggaccgactaatgaatccactcatcgaccaatacttgtactatctctcaaagactattaacggttctggacagaatcaacaaacgctaaaattcagtgtggccggacccagcaacatggctgtccagggaagaaactacatacctggacccagctaccgacaacaacgtgtctcaaccactgtgactcaaaacaacaacagcgaatttgcttggcctggagcttcttcttgggctctcaatggacgtaatagcttgatgaatcctggacctgctatggccagccacaaagaaggagaggaccgtttctttcctttgtctggatctttaatttttggcaaacaaggaactggaagagacaacgtggatgcggacaaagtcatgataaccaacgaagaagaaattaaaactactaacccggtagcaacggagtcctatggacaagtggccacaaaccaccagggccagagtggccgcggcgatctgggcctgagcgcccaggcggcccagaccggctgggttcaaaaccaaggaatacttccgggtatggtttggcaggacagagatgtgtacctgcaaggacccatttgggccaaaattcctcacacggacggcaactttcacccttctccgctgatgggagggtttggaatgaaacacccgcctcctcagatcctcatcaaaaacacacctgtacctgcggatcctccaacggccttcaacaaggacaagctgaactctttcatcacccagtattctactggccaagtcagcgtggagatcgagtgggagctgcagaaggaaaacagcaagcgctggaacccggagatccagtacacttccaactattacaagtctaataatgttgaatttgctgttaatactgaaggtgtatatagtgaaccccgccccattggcaccagatacctgactcgtaatctgtaa

SEQ ID NO: 14 - protein, 745 aa, synthetic construct
  REGION 1..745: note = AAV9LD_P1 capsid polypeptide, insertion site 588
MAADGYLPDWLEDNLSEGIREWWALKPGAPQPKANQQHQDNARGLVLPGYKYLGPGNGLDKGEPVNAADAAALEHDKAYDQQLKAGDNPYLKYNHADAEFQERLKEDTSFGGNLGRAVFQAKKRLLEPLGLVEEAAKTAPGKKRPVEQSPQEPDSSAGIGKSGAQPAKKRLNFGQTGDTESVPDPQPIGEPPAAPSGVGSLTMASGGGAPVADNNEGADGVGSSSGNWHCDSQWLGDRVITTSTRTWALPTYNNHLYKQISNSTSGGSSNDNAYFGYSTPWGYFDFNRFHCHFSPRDWQRLINNNWGFRPKRLNFKLFNIQVKEVTDNNGVKTIANNLTSTVQVFTDSDYQLPYVLGSAHEGCLPPFPADVFMIPQYGYLTLNDGSQAVGRSSFYCLEYFPSQMLRTGNNFQFSYEFENVPFHSSYAHSQSLDRLMNPLIDQYLYYLSKTINGSGQNQQTLKFSVAGPSNMAVQGRNYIPGPSYRQQRVSTTVTQNNNSEFAWAAASSWALNGRNSLMNPGPAMASHKEGEDRFFPLSGSLIFGKQGTGRDNVDADKVMITNEEEIKTTNPVATESYGQVATNHQGQSGRGDLGLSAQAAQTGWVQNQGILPGMVWQDRDVYLQGPIWAKIPHTDGNFHPSPLMGGFGMKHPPPQILIKNTPVPADPPTAFNKDKLNSFITQYSTGQVSVEIEWELQKENSKRWNPEIQYTSNYYKSNNVEFAVNTEGVYSEPRPIGTRYLTRNL

SEQ ID NO: 15 - DNA, 2238 bp, synthetic construct
  misc_feature 1..2238: note = AAV9LD_P1 capsid polypeptide encoding, insertion site amino acid 588
  source 1..2238: mol_type = other DNA
atggctgccgatggttatcttccagattggctcgaggacaaccttagtgaaggaattcgcgagtggtgggctttgaaacctggagcccctcaacccaaggcaaatcaacaacatcaagacaacgctcgaggtcttgtgcttccgggttacaaataccttggacccggcaacggactcgacaagggggagccggtcaacgcagcagacgcggcggccctcgagcacgacaaggcctacgaccagcagctcaaggccggagacaacccgtacctcaagtacaaccacgccgacgccgagttccaggagcggctcaaagaagatacgtcttttgggggcaacctcgggcgagcagtcttccaggccaaaaagaggcttcttgaacctcttggtctggttgaggaagcggctaagacggctcctggaaagaagaggcctgtagagcagtctcctcaggaaccggactcctccgcgggtattggcaaatcgggtgcacagcccgctaaaaagagactcaatttcggtcagactggcgacacagagtcagtcccagaccctcaaccaatcggagaacctcccgcagccccctcaggtgtgggatctcttacaatggcttcaggtggtggcgcaccagtggcagacaataacgaaggtgccgatggagtgggtagttcctcgggaaattggcattgcgattcccaatggctgggggacagagtcatcaccaccagcacccgaacctgggccctgcccacctacaacaatcacctctacaagcaaatctccaacagcacatctggaggatcttcaaatgacaacgcctacttcggctacagcaccccctgggggtattttgacttcaacagattccactgccacttctcaccacgtgactggcagcgactcatcaacaacaactggggattccggcctaagcgactcaacttcaagctcttcaacattcaggtcaaagaggttacggacaacaatggagtcaagaccatcgccaataaccttaccagcacggtccaggtcttcacggactcagactatcagctcccgtacgtgctcgggtcggctcacgagggctgcctcccgccgttcccagcggacgttttcatgattcctcagtacgggtatctgacgcttaatgatggaagccaggccgtgggtcgttcgtccttttactgcctggaatatttcccgtcgcaaatgctaagaacgggtaacaacttccagttcagctacgagtttgagaacgtacctttccatagcagctacgctcacagccaaagcctggaccgactaatgaatccactcatcgaccaatacttgtactatctctcaaagactattaacggttctggacagaatcaacaaacgctaaaattcagtgtggccggacccagcaacatggctgtccagggaagaaactacatacctggacccagctaccgacaacaacgtgtctcaaccactgtgactcaaaacaacaacagcgaatttgcttgggctgcagcttcttcttgggctctcaatggacgtaatagcttgatgaatcctggacctgctatggccagccacaaagaaggagaggaccgtttctttcctttgtctggatctttaatttttggcaaacaaggaactggaagagacaacgtggatgcggacaaagtcatgataaccaacgaagaagaaattaaaactactaacccggtagcaacggagtcctatggacaagtggccacaaaccaccagggccagagtggccgcggcgatctgggcctgagcgcccaggcggcccagaccggctgggttcaaaaccaaggaatacttccgggtatggtttggcaggacagagatgtgtacctgcaaggacccatttgggccaaaattcctcacacggacggcaactttcacccttctccgctgatgggagggtttggaatgaaacacccgcctcctcagatcctcatcaaaaacacacctgtacctgcggatcctccaacggccttcaacaaggacaagctgaactctttcatcacccagtattctactggccaagtcagcgtggagatcgagtgggagctgcagaaggaaaacagcaagcgctggaacccggagatccagtacacttccaactattacaagtctaataatgttgaatttgctgttaatactgaaggtgtatatagtgaaccccgccccattggcaccagatacctgactcgtaatctgtaa

SEQ ID NO: 16 - protein, 745 aa, synthetic construct
  REGION 1..745: note = AAV9_P1 capsid polypeptide, insertion site 589
MAADGYLPDWLEDNLSEGIREWWALKPGAPQPKANQQHQDNARGLVLPGYKYLGPGNGLDKGEPVNAADAAALEHDKAYDQQLKAGDNPYLKYNHADAEFQERLKEDTSFGGNLGRAVFQAKKRLLEPLGLVEEAAKTAPGKKRPVEQSPQEPDSSAGIGKSGAQPAKKRLNFGQTGDTESVPDPQPIGEPPAAPSGVGSLTMASGGGAPVADNNEGADGVGSSSGNWHCDSQWLGDRVITTSTRTWALPTYNNHLYKQISNSTSGGSSNDNAYFGYSTPWGYFDFNRFHCHFSPRDWQRLINNNWGFRPKRLNFKLFNIQVKEVTDNNGVKTIANNLTSTVQVFTDSDYQLPYVLGSAHEGCLPPFPADVFMIPQYGYLTLNDGSQAVGRSSFYCLEYFPSQMLRTGNNFQFSYEFENVPFHSSYAHSQSLDRLMNPLIDQYLYYLSKTINGSGQNQQTLKFSVAGPSNMAVQGRNYIPGPSYRQQRVSTTVTQNNNSEFAWPGASSWALNGRNSLMNPGPAMASHKEGEDRFFPLSGSLIFGKQGTGRDNVDADKVMITNEEEIKTTNPVATESYGQVATNHQSGQSGRGDLGLSAQAATGWVQNQGILPGMVWQDRDVYLQGPIWAKIPHTDGNFHPSPLMGGFGMKHPPPQILIKNTPVPADPPTAFNKDKLNSFITQYSTGQVSVEIEWELQKENSKRWNPEIQYTSNYYKSNNVEFAVNTEGVYSEPRPIGTRYLTRNL

SEQ ID NO: 17 - DNA, 2238 bp, synthetic construct
  misc_feature 1..2238: note = AAV9_P1 capsid polypeptide 2 encoding, insertion site amino acid 589
  source 1..2238: mol_type = other DNA
atggctgccgatggttatcttccagattggctcgaggacaaccttagtgaaggaattcgcgagtggtgggctttgaaacctggagcccctcaacccaaggcaaatcaacaacatcaagacaacgctcgaggtcttgtgcttccgggttacaaataccttggacccggcaacggactcgacaagggggagccggtcaacgcagcagacgcggcggccctcgagcacgacaaggcctacgaccagcagctcaaggccggagacaacccgtacctcaagtacaaccacgccgacgccgagttccaggagcggctcaaagaagatacgtcttttgggggcaacctcgggcgagcagtcttccaggccaaaaagaggcttcttgaacctcttggtctggttgaggaagcggctaagacggctcctggaaagaagaggcctgtagagcagtctcctcaggaaccggactcctccgcgggtattggcaaatcgggtgcacagcccgctaaaaagagactcaatttcggtcagactggcgacacagagtcagtcccagaccctcaaccaatcggagaacctcccgcagccccctcaggtgtgggatctcttacaatggcttcaggtggtggcgcaccagtggcagacaataacgaaggtgccgatggagtgggtagttcctcgggaaattggcattgcgattcccaatggctgggggacagagtcatcaccaccagcacccgaacctgggccctgcccacctacaacaatcacctctacaagcaaatctccaacagcacatctggaggatcttcaaatgacaacgcctacttcggctacagcaccccctgggggtattttgacttcaacagattccactgccacttctcaccacgtgactggcagcgactcatcaacaacaactggggattccggcctaagcgactcaacttcaagctcttcaacattcaggtcaaagaggttacggacaacaatggagtcaagaccatcgccaataaccttaccagcacggtccaggtcttcacggactcagactatcagctcccgtacgtgctcgggtcggctcacgagggctgcctcccgccgttcccagcggacgttttcatgattcctcagtacgggtatctgacgcttaatgatggaagccaggccgtgggtcgttcgtccttttactgcctggaatatttcccgtcgcaaatgctaagaacgggtaacaacttccagttcagctacgagtttgagaacgtacctttccatagcagctacgctcacagccaaagcctggaccgactaatgaatccactcatcgaccaatacttgtactatctctcaaagactattaacggttctggacagaatcaacaaacgctaaaattcagtgtggccggacccagcaacatggctgtccagggaagaaactacatacctggacccagctaccgacaacaacgtgtctcaaccactgtgactcaaaacaacaacagcgaatttgcttggcctggagcttcttcttgggctctcaatggacgtaatagcttgatgaatcctggacctgctatggccagccacaaagaaggagaggaccgtttctttcctttgtctggatctttaatttttggcaaacaaggaactggaagagacaacgtggatgcggacaaagtcatgataaccaacgaagaagaaattaaaactactaacccggtagcaacggagtcctatggacaagtggccacaaaccaccagagtggccagagtggccgcggcgatctgggcctgagcgcccaggcggccaccggctgggttcaaaaccaaggaatacttccgggtatggtttggcaggacagagatgtgtacctgcaaggacccatttgggccaaaattcctcacacggacggcaactttcacccttctccgctgatgggagggtttggaatgaaacacccgcctcctcagatcctcatcaaaaacacacctgtacctgcggatcctccaacggccttcaacaaggacaagctgaactctttcatcacccagtattctactggccaagtcagcgtggagatcgagtgggagctgcagaaggaaaacagcaagcgctggaacccggagatccagtacacttccaactattacaagtctaataatgttgaatttgctgttaatactgaaggtgtatatagtgaaccccgccccattggcaccagatacctgactcgtaatctgtaa

SEQ ID NO: 18 - protein, 745 aa, synthetic construct
  REGION 1..745: note = AAV9_P3 capsid polypeptide, insertion site 588
MAADGYLPDWLEDNLSEGIREWWALKPGAPQPKANQQHQDNARGLVLPGYKYLGPGNGLDKGEPVNAADAAALEHDKAYDQQLKAGDNPYLKYNHADAEFQERLKEDTSFGGNLGRAVFQAKKRLLEPLGLVEEAAKTAPGKKRPVEQSPQEPDSSAGIGKSGAQPAKKRLNFGQTGDTESVPDPQPIGEPPAAPSGVGSLTMASGGGAPVADNNEGADGVGSSSGNWHCDSQWLGDRVITTSTRTWALPTYNNHLYKQISNSTSGGSSNDNAYFGYSTPWGYFDFNRFHCHFSPRDWQRLINNNWGFRPKRLNFKLFNIQVKEVTDNNGVKTIANNLTSTVQVFTDSDYQLPYVLGSAHEGCLPPFPADVFMIPQYGYLTLNDGSQAVGRSSFYCLEYFPSQMLRTGNNFQFSYEFENVPFHSSYAHSQSLDRLMNPLIDQYLYYLSKTINGSGQNQQTLKFSVAGPSNMAVQGRNYIPGPSYRQQRVSTTVTQNNNSEFAWPGASSWALNGRNSLMNPGPAMASHKEGEDRFFPLSGSLIFGKQGTGRDNVDADKVMITNEEEIKTTNPVATESYGQVATNHQGQSGRGDAVGVAQAAQTGWVQNQGILPGMVWQDRDVYLQGPIWAKIPHTDGNFHPSPLMGGFGMKHPPPQILIKNTPVPADPPTAFNKDKLNSFITQYSTGQVSVEIEWELQKENSKRWNPEIQYTSNYYKSNNVEFAVNTEGVYSEPRPIGTRYLTRNL

SEQ ID NO: 19 - DNA, 2238 bp, synthetic construct
  misc_feature 1..2238: note = AAV9_P3 capsid polypeptide encoding, insertion site 588
  source 1..2238: mol_type = other DNA
atggctgccgatggttatcttccagattggctcgaggacaaccttagtgaaggaattcgcgagtggtgggctttgaaacctggagcccctcaacccaaggcaaatcaacaacatcaagacaacgctcgaggtcttgtgcttccgggttacaaataccttggacccggcaacggactcgacaagggggagccggtcaacgcagcagacgcggcggccctcgagcacgacaaggcctacgaccagcagctcaaggccggagacaacccgtacctcaagtacaaccacgccgacgccgagttccaggagcggctcaaagaagatacgtcttttgggggcaacctcgggcgagcagtcttccaggccaaaaagaggcttcttgaacctcttggtctggttgaggaagcggctaagacggctcctggaaagaagaggcctgtagagcagtctcctcaggaaccggactcctccgcgggtattggcaaatcgggtgcacagcccgctaaaaagagactcaatttcggtcagactggcgacacagagtcagtcccagaccctcaaccaatcggagaacctcccgcagccccctcaggtgtgggatctcttacaatggcttcaggtggtggcgcaccagtggcagacaataacgaaggtgccgatggagtgggtagttcctcgggaaattggcattgcgattcccaatggctgggggacagagtcatcaccaccagcacccgaacctgggccctgcccacctacaacaatcacctctacaagcaaatctccaacagcacatctggaggatcttcaaatgacaacgcctacttcggctacagcaccccctgggggtattttgacttcaacagattccactgccacttctcaccacgtgactggcagcgactcatcaacaacaactggggattccggcctaagcgactcaacttcaagctcttcaacattcaggtcaaagaggttacggacaacaatggagtcaagaccatcgccaataaccttaccagcacggtccaggtcttcacggactcagactatcagctcccgtacgtgctcgggtcggctcacgagggctgcctcccgccgttcccagcggacgttttcatgattcctcagtacgggtatctgacgcttaatgatggaagccaggccgtgggtcgttcgtccttttactgcctggaatatttcccgtcgcaaatgctaagaacgggtaacaacttccagttcagctacgagtttgagaacgtacctttccatagcagctacgctcacagccaaagcctggaccgactaatgaatccactcatcgaccaatacttgtactatctctcaaagactattaacggttctggacagaatcaacaaacgctaaaattcagtgtggccggacccagcaacatggctgtccagggaagaaactacatacctggacccagctaccgacaacaacgtgtctcaaccactgtgactcaaaacaacaacagcgaatttgcttggcctggagcttcttcttgggctctcaatggacgtaatagcttgatgaatcctggacctgctatggccagccacaaagaaggagaggaccgtttctttcctttgtctggatctttaatttttggcaaacaaggaactggaagagacaacgtggatgcggacaaagtcatgataaccaacgaagaagaaattaaaactactaacccggtagcaacggagtcctatggacaagtggccacaaaccaccagggccagagtggccgcggcgatgcggtgggcgtggcccaggcggcccagaccggctgggttcaaaaccaaggaatacttccgggtatggtttggcaggacagagatgtgtacctgcaaggacccatttgggccaaaattcctcacacggacggcaactttcacccttctccgctgatgggagggtttggaatgaaacacccgcctcctcagatcctcatcaaaaacacacctgtacctgcggatcctccaacggccttcaacaaggacaagctgaactctttcatcacccagtattctactggccaagtcagcgtggagatcgagtgggagctgcagaaggaaaacagcaagcgctggaacccggagatccagtacacttccaactattacaagtctaataatgttgaatttgctgttaatactgaaggtgtatatagtgaaccccgccccattggcaccagatacctgactcgtaatctgtaa

SEQ ID NO: 20 - protein, 745 aa, synthetic construct
  REGION 1..745: note = AAV9_P3 capsid polypeptide 2, insertion site 589
MAADGYLPDWLEDNLSEGIREWWALKPGAPQPKANQQHQDNARGLVLPGYKYLGPGNGLDKGEPVNAADAAALEHDKAYDQQLKAGDNPYLKYNHADAEFQERLKEDTSFGGNLGRAVFQAKKRLLEPLGLVEEAAKTAPGKKRPVEQSPQEPDSSAGIGKSGAQPAKKRLNFGQTGDTESVPDPQPIGEPPAAPSGVGSLTMASGGGAPVADNNEGADGVGSSSGNWHCDSQWLGDRVITTSTRTWALPTYNNHLYKQISNSTSGGSSNDNAYFGYSTPWGYFDFNRFHCHFSPRDWQRLINNNWGFRPKRLNFKLFNIQVKEVTDNNGVKTIANNLTSTVQVFTDSDYQLPYVLGSAHEGCLPPFPADVFMIPQYGYLTLNDGSQAVGRSSFYCLEYFPSQMLRTGNNFQFSYEFENVPFHSSYAHSQSLDRLMNPLIDQYLYYLSKTINGSGQNQQTLKFSVAGPSNMAVQGRNYIPGPSYRQQRVSTTVTQNNNSEFAWPGASSWALNGRNSLMNPGPAMASHKEGEDRFFPLSGSLIFGKQGTGRDNVDADKVMITNEEEIKTTNPVATESYGQVATNHQSGQSGRGDAVGVAQAATGWVQNQGILPGMVWQDRDVYLQGPIWAKIPHTDGNFHPSPLMGGFGMKHPPPQILIKNTPVPADPPTAFNKDKLNSFITQYSTGQVSVEIEWELQKENSKRWNPEIQYTSNYYKSNNVEFAVNTEGVYSEPRPIGTRYLTRNL

SEQ ID NO: 21 - DNA, 2238 bp, synthetic construct
  misc_feature 1..2238: note = AAV9_P3 capsid polypeptide 2 encoding, insertion site 589
  source 1..2238: mol_type = other DNA
atggctgccgatggttatcttccagattggctcgaggacaaccttagtgaaggaattcgcgagtggtgggctttgaaacctggagcccctcaacccaaggcaaatcaacaacatcaagacaacgctcgaggtcttgtgcttccgggttacaaataccttggacccggcaacggactcgacaagggggagccggtcaacgcagcagacgcggcggccctcgagcacgacaaggcctacgaccagcagctcaaggccggagacaacccgtacctcaagtacaaccacgccgacgccgagttccaggagcggctcaaagaagatacgtcttttgggggcaacctcgggcgagcagtcttccaggccaaaaagaggcttcttgaacctcttggtctggttgaggaagcggctaagacggctcctggaaagaagaggcctgtagagcagtctcctcaggaaccggactcctccgcgggtattggcaaatcgggtgcacagcccgctaaaaagagactcaatttcggtcagactggcgacacagagtcagtcccagaccctcaaccaatcggagaacctcccgcagccccctcaggtgtgggatctcttacaatggcttcaggtggtggcgcaccagtggcagacaataacgaaggtgccgatggagtgggtagttcctcgggaaattggcattgcgattcccaatggctgggggacagagtcatcaccaccagcacccgaacctgggccctgcccacctacaacaatcacctctacaagcaaatctccaacagcacatctggaggatcttcaaatgacaacgcctacttcggctacagcaccccctgggggtattttgacttcaacagattccactgccacttctcaccacgtgactggcagcgactcatcaacaacaactggggattccggcctaagcgactcaacttcaagctcttcaacattcaggtcaaagaggttacggacaacaatggagtcaagaccatcgccaataaccttaccagcacggtccaggtcttcacggactcagactatcagctcccgtacgtgctcgggtcggctcacgagggctgcctcccgccgttcccagcggacgttttcatgattcctcagtacgggtatctgacgcttaatgatggaagccaggccgtgggtcgttcgtccttttactgcctggaatatttcccgtcgcaaatgctaagaacgggtaacaacttccagttcagctacgagtttgagaacgtacctttccatagcagctacgctcacagccaaagcctggaccgactaatgaatccactcatcgaccaatacttgtactatctctcaaagactattaacggttctggacagaatcaacaaacgctaaaattcagtgtggccggacccagcaacatggctgtccagggaagaaactacatacctggacccagctaccgacaacaacgtgtctcaaccactgtgactcaaaacaacaacagcgaatttgcttggcctggagcttcttcttgggctctcaatggacgtaatagcttgatgaatcctggacctgctatggccagccacaaagaaggagaggaccgtttctttcctttgtctggatctttaatttttggcaaacaaggaactggaagagacaacgtggatgcggacaaagtcatgataaccaacgaagaagaaattaaaactactaacccggtagcaacggagtcctatggacaagtggccacaaaccaccagagtggccagagtggccgcggcgatgcggtgggcgtggcccaggcggccaccggctgggttcaaaaccaaggaatacttccgggtatggtttggcaggacagagatgtgtacctgcaaggacccatttgggccaaaattcctcacacggacggcaactttcacccttctccgctgatgggagggtttggaatgaaacacccgcctcctcagatcctcatcaaaaacacacctgtacctgcggatcctccaacggccttcaacaaggacaagctgaactctttcatcacccagtattctactggccaagtcagcgtggagatcgagtgggagctgcagaaggaaaacagcaagcgctggaacccggagatccagtacacttccaactattacaagtctaataatgttgaatttgctgttaatactgaaggtgtatatagtgaaccccgccccattggcaccagatacctgactcgtaatctgtaa

SEQ ID NO: 22 - protein, 745 aa, synthetic construct
  REGION 1..745: note = AAV9LD_P1 capsid polypeptide 2, insertion site 589
MAADGYLPDWLEDNLSEGIREWWALKPGAPQPKANQQHQDNARGLVLPGYKYLGPGNGLDKGEPVNAADAAALEHDKAYDQQLKAGDNPYLKYNHADAEFQERLKEDTSFGGNLGRAVFQAKKRLLEPLGLVEEAAKTAPGKKRPVEQSPQEPDSSAGIGKSGAQPAKKRLNFGQTGDTESVPDPQPIGEPPAAPSGVGSLTMASGGGAPVADNNEGADGVGSSSGNWHCDSQWLGDRVITTSTRTWALPTYNNHLYKQISNSTSGGSSNDNAYFGYSTPWGYFDFNRFHCHFSPRDWQRLINNNWGFRPKRLNFKLFNIQVKEVTDNNGVKTIANNLTSTVQVFTDSDYQLPYVLGSAHEGCLPPFPADVFMIPQYGYLTLNDGSQAVGRSSFYCLEYFPSQMLRTGNNFQFSYEFENVPFHSSYAHSQSLDRLMNPLIDQYLYYLSKTINGSGQNQQTLKFSVAGPSNMAVQGRNYIPGPSYRQQRVSTTVTQNNNSEFAWAAASSWALNGRNSLMNPGPAMASHKEGEDRFFPLSGSLIFGKQGTGRDNVDADKVMITNEEEIKTTNPVATESYGQVATNHQSGQSGRGDLGLSAQAATGWVQNQGILPGMVWQDRDVYLQGPIWAKIPHTDGNFHPSPLMGGFGMKHPPPQILIKNTPVPADPPTAFNKDKLNSFITQYSTGQVSVEIEWELQKENSKRWNPEIQYTSNYYKSNNVEFAVNTEGVYSEPRPIGTRYLTRNL

SEQ ID NO: 23 - DNA, 2238 bp, synthetic construct
  misc_feature 1..2238: note = AAV9LD_P1 capsid polypeptide 2 encoding, insertion site amno acid 589
  source 1..2238: mol_type = other DNA
atggctgccgatggttatcttccagattggctcgaggacaaccttagtgaaggaattcgcgagtggtgggctttgaaacctggagcccctcaacccaaggcaaatcaacaacatcaagacaacgctcgaggtcttgtgcttccgggttacaaataccttggacccggcaacggactcgacaagggggagccggtcaacgcagcagacgcggcggccctcgagcacgacaaggcctacgaccagcagctcaaggccggagacaacccgtacctcaagtacaaccacgccgacgccgagttccaggagcggctcaaagaagatacgtcttttgggggcaacctcgggcgagcagtcttccaggccaaaaagaggcttcttgaacctcttggtctggttgaggaagcggctaagacggctcctggaaagaagaggcctgtagagcagtctcctcaggaaccggactcctccgcgggtattggcaaatcgggtgcacagcccgctaaaaagagactcaatttcggtcagactggcgacacagagtcagtcccagaccctcaaccaatcggagaacctcccgcagccccctcaggtgtgggatctcttacaatggcttcaggtggtggcgcaccagtggcagacaataacgaaggtgccgatggagtgggtagttcctcgggaaattggcattgcgattcccaatggctgggggacagagtcatcaccaccagcacccgaacctgggccctgcccacctacaacaatcacctctacaagcaaatctccaacagcacatctggaggatcttcaaatgacaacgcctacttcggctacagcaccccctgggggtattttgacttcaacagattccactgccacttctcaccacgtgactggcagcgactcatcaacaacaactggggattccggcctaagcgactcaacttcaagctcttcaacattcaggtcaaagaggttacggacaacaatggagtcaagaccatcgccaataaccttaccagcacggtccaggtcttcacggactcagactatcagctcccgtacgtgctcgggtcggctcacgagggctgcctcccgccgttcccagcggacgttttcatgattcctcagtacgggtatctgacgcttaatgatggaagccaggccgtgggtcgttcgtccttttactgcctggaatatttcccgtcgcaaatgctaagaacgggtaacaacttccagttcagctacgagtttgagaacgtacctttccatagcagctacgctcacagccaaagcctggaccgactaatgaatccactcatcgaccaatacttgtactatctctcaaagactattaacggttctggacagaatcaacaaacgctaaaattcagtgtggccggacccagcaacatggctgtccagggaagaaactacatacctggacccagctaccgacaacaacgtgtctcaaccactgtgactcaaaacaacaacagcgaatttgcttgggctgcagcttcttcttgggctctcaatggacgtaatagcttgatgaatcctggacctgctatggccagccacaaagaaggagaggaccgtttctttcctttgtctggatctttaatttttggcaaacaaggaactggaagagacaacgtggatgcggacaaagtcatgataaccaacgaagaagaaattaaaactactaacccggtagcaacggagtcctatggacaagtggccacaaaccaccagagtggccagagtggccgcggcgatctgggcctgagcgcccaggcggccaccggctgggttcaaaaccaaggaatacttccgggtatggtttggcaggacagagatgtgtacctgcaaggacccatttgggccaaaattcctcacacggacggcaactttcacccttctccgctgatgggagggtttggaatgaaacacccgcctcctcagatcctcatcaaaaacacacctgtacctgcggatcctccaacggccttcaacaaggacaagctgaactctttcatcacccagtattctactggccaagtcagcgtggagatcgagtgggagctgcagaaggaaaacagcaagcgctggaacccggagatccagtacacttccaactattacaagtctaataatgttgaatttgctgttaatactgaaggtgtatatagtgaaccccgccccattggcaccagatacctgactcgtaatctgtaa

SEQ ID NO: 24 - protein, 745 aa, synthetic construct
  REGION 1..745: note = AAV9LD_P3 capsid polypeptide, insertion site 588
MAADGYLPDWLEDNLSEGIREWWALKPGAPQPKANQQHQDNARGLVLPGYKYLGPGNGLDKGEPVNAADAAALEHDKAYDQQLKAGDNPYLKYNHADAEFQERLKEDTSFGGNLGRAVFQAKKRLLEPLGLVEEAAKTAPGKKRPVEQSPQEPDSSAGIGKSGAQPAKKRLNFGQTGDTESVPDPQPIGEPPAAPSGVGSLTMASGGGAPVADNNEGADGVGSSSGNWHCDSQWLGDRVITTSTRTWALPTYNNHLYKQISNSTSGGSSNDNAYFGYSTPWGYFDFNRFHCHFSPRDWQRLINNNWGFRPKRLNFKLFNIQVKEVTDNNGVKTIANNLTSTVQVFTDSDYQLPYVLGSAHEGCLPPFPADVFMIPQYGYLTLNDGSQAVGRSSFYCLEYFPSQMLRTGNNFQFSYEFENVPFHSSYAHSQSLDRLMNPLIDQYLYYLSKTINGSGQNQQTLKFSVAGPSNMAVQGRNYIPGPSYRQQRVSTTVTQNNNSEFAWAAASSWALNGRNSLMNPGPAMASHKEGEDRFFPLSGSLIFGKQGTGRDNVDADKVMITNEEEIKTTNPVATESYGQVATNHQGQSGRGDAVGVAQAAQTGWVQNQGILPGMVWQDRDVYLQGPIWAKIPHTDGNFHPSPLMGGFGMKHPPPQILIKNTPVPADPPTAFNKDKLNSFITQYSTGQVSVEIEWELQKENSKRWNPEIQYTSNYYKSNNVEFAVNTEGVYSEPRPIGTRYLTRNL

SEQ ID NO: 25 - DNA, 2238 bp, synthetic construct
  misc_feature 1..2238: note = AAV9LD_P3 capsid polypeptide encoding, insertion site amino acid 588
  source 1..2238: mol_type = other DNA
atggctgccgatggttatcttccagattggctcgaggacaaccttagtgaaggaattcgcgagtggtgggctttgaaacctggagcccctcaacccaaggcaaatcaacaacatcaagacaacgctcgaggtcttgtgcttccgggttacaaataccttggacccggcaacggactcgacaagggggagccggtcaacgcagcagacgcggcggccctcgagcacgacaaggcctacgaccagcagctcaaggccggagacaacccgtacctcaagtacaaccacgccgacgccgagttccaggagcggctcaaagaagatacgtcttttgggggcaacctcgggcgagcagtcttccaggccaaaaagaggcttcttgaacctcttggtctggttgaggaagcggctaagacggctcctggaaagaagaggcctgtagagcagtctcctcaggaaccggactcctccgcgggtattggcaaatcgggtgcacagcccgctaaaaagagactcaatttcggtcagactggcgacacagagtcagtcccagaccctcaaccaatcggagaacctcccgcagccccctcaggtgtgggatctcttacaatggcttcaggtggtggcgcaccagtggcagacaataacgaaggtgccgatggagtgggtagttcctcgggaaattggcattgcgattcccaatggctgggggacagagtcatcaccaccagcacccgaacctgggccctgcccacctacaacaatcacctctacaagcaaatctccaacagcacatctggaggatcttcaaatgacaacgcctacttcggctacagcaccccctgggggtattttgacttcaacagattccactgccacttctcaccacgtgactggcagcgactcatcaacaacaactggggattccggcctaagcgactcaacttcaagctcttcaacattcaggtcaaagaggttacggacaacaatggagtcaagaccatcgccaataaccttaccagcacggtccaggtcttcacggactcagactatcagctcccgtacgtgctcgggtcggctcacgagggctgcctcccgccgttcccagcggacgttttcatgattcctcagtacgggtatctgacgcttaatgatggaagccaggccgtgggtcgttcgtccttttactgcctggaatatttcccgtcgcaaatgctaagaacgggtaacaacttccagttcagctacgagtttgagaacgtacctttccatagcagctacgctcacagccaaagcctggaccgactaatgaatccactcatcgaccaatacttgtactatctctcaaagactattaacggttctggacagaatcaacaaacgctaaaattcagtgtggccggacccagcaacatggctgtccagggaagaaactacatacctggacccagctaccgacaacaacgtgtctcaaccactgtgactcaaaacaacaacagcgaatttgcttgggctgcagcttcttcttgggctctcaatggacgtaatagcttgatgaatcctggacctgctatggccagccacaaagaaggagaggaccgtttctttcctttgtctggatctttaatttttggcaaacaaggaactggaagagacaacgtggatgcggacaaagtcatgataaccaacgaagaagaaattaaaactactaacccggtagcaacggagtcctatggacaagtggccacaaaccaccagggccagagtggccgcggcgatgcggtgggcgtggcccaggcggcccagaccggctgggttcaaaaccaaggaatacttccgggtatggtttggcaggacagagatgtgtacctgcaaggacccatttgggccaaaattcctcacacggacggcaactttcacccttctccgctgatgggagggtttggaatgaaacacccgcctcctcagatcctcatcaaaaacacacctgtacctgcggatcctccaacggccttcaacaaggacaagctgaactctttcatcacccagtattctactggccaagtcagcgtggagatcgagtgggagctgcagaaggaaaacagcaagcgctggaacccggagatccagtacacttccaactattacaagtctaataatgttgaatttgctgttaatactgaaggtgtatatagtgaaccccgccccattggcaccagatacctgactcgtaatctgtaa

SEQ ID NO: 26 - protein, 745 aa, synthetic construct
  REGION 1..745: note = AAV9LD_P3 capsid polypeptide 2, insertion site 589
MAADGYLPDWLEDNLSEGIREWWALKPGAPQPKANQQHQDNARGLVLPGYKYLGPGNGLDKGEPVNAADAAALEHDKAYDQQLKAGDNPYLKYNHADAEFQERLKEDTSFGGNLGRAVFQAKKRLLEPLGLVEEAAKTAPGKKRPVEQSPQEPDSSAGIGKSGAQPAKKRLNFGQTGDTESVPDPQPIGEPPAAPSGVGSLTMASGGGAPVADNNEGADGVGSSSGNWHCDSQWLGDRVITTSTRTWALPTYNNHLYKQISNSTSGGSSNDNAYFGYSTPWGYFDFNRFHCHFSPRDWQRLINNNWGFRPKRLNFKLFNIQVKEVTDNNGVKTIANNLTSTVQVFTDSDYQLPYVLGSAHEGCLPPFPADVFMIPQYGYLTLNDGSQAVGRSSFYCLEYFPSQMLRTGNNFQFSYEFENVPFHSSYAHSQSLDRLMNPLIDQYLYYLSKTINGSGQNQQTLKFSVAGPSNMAVQGRNYIPGPSYRQQRVSTTVTQNNNSEFAWAAASSWALNGRNSLMNPGPAMASHKEGEDRFFPLSGSLIFGKQGTGRDNVDADKVMITNEEEIKTTNPVATESYGQVATNHQSGQSGRGDAVGVAQAATGWVQNQGILPGMVWQDRDVYLQGPIWAKIPHTDGNFHPSPLMGGFGMKHPPPQILIKNTPVPADPPTAFNKDKLNSFITQYSTGQVSVEIEWELQKENSKRWNPEIQYTSNYYKSNNVEFAVNTEGVYSEPRPIGTRYLTRNL

SEQ ID NO: 27 - DNA, 2238 bp, synthetic construct
  misc_feature 1..2238: note = AAV9LD_P3 capsid polypeptide 2 encoding, insertion site amino acid 589
  source 1..2238: mol_type = other DNA
atggctgccgatggttatcttccagattggctcgaggacaaccttagtgaaggaattcgcgagtggtgggctttgaaacctggagcccctcaacccaaggcaaatcaacaacatcaagacaacgctcgaggtcttgtgcttccgggttacaaataccttggacccggcaacggactcgacaagggggagccggtcaacgcagcagacgcggcggccctcgagcacgacaaggcctacgaccagcagctcaaggccggagacaacccgtacctcaagtacaaccacgccgacgccgagttccaggagcggctcaaagaagatacgtcttttgggggcaacctcgggcgagcagtcttccaggccaaaaagaggcttcttgaacctcttggtctggttgaggaagcggctaagacggctcctggaaagaagaggcctgtagagcagtctcctcaggaaccggactcctccgcgggtattggcaaatcgggtgcacagcccgctaaaaagagactcaatttcggtcagactggcgacacagagtcagtcccagaccctcaaccaatcggagaacctcccgcagccccctcaggtgtgggatctcttacaatggcttcaggtggtggcgcaccagtggcagacaataacgaaggtgccgatggagtgggtagttcctcgggaaattggcattgcgattcccaatggctgggggacagagtcatcaccaccagcacccgaacctgggccctgcccacctacaacaatcacctctacaagcaaatctccaacagcacatctggaggatcttcaaatgacaacgcctacttcggctacagcaccccctgggggtattttgacttcaacagattccactgccacttctcaccacgtgactggcagcgactcatcaacaacaactggggattccggcctaagcgactcaacttcaagctcttcaacattcaggtcaaagaggttacggacaacaatggagtcaagaccatcgccaataaccttaccagcacggtccaggtcttcacggactcagactatcagctcccgtacgtgctcgggtcggctcacgagggctgcctcccgccgttcccagcggacgttttcatgattcctcagtacgggtatctgacgcttaatgatggaagccaggccgtgggtcgttcgtccttttactgcctggaatatttcccgtcgcaaatgctaagaacgggtaacaacttccagttcagctacgagtttgagaacgtacctttccatagcagctacgctcacagccaaagcctggaccgactaatgaatccactcatcgaccaatacttgtactatctctcaaagactattaacggttctggacagaatcaacaaacgctaaaattcagtgtggccggacccagcaacatggctgtccagggaagaaactacatacctggacccagctaccgacaacaacgtgtctcaaccactgtgactcaaaacaacaacagcgaatttgcttgggctgcagcttcttcttgggctctcaatggacgtaatagcttgatgaatcctggacctgctatggccagccacaaagaaggagaggaccgtttctttcctttgtctggatctttaatttttggcaaacaaggaactggaagagacaacgtggatgcggacaaagtcatgataaccaacgaagaagaaattaaaactactaacccggtagcaacggagtcctatggacaagtggccacaaaccaccagagtggccagagtggccgcggcgatgcggtgggcgtggcccaggcggccaccggctgggttcaaaaccaaggaatacttccgggtatggtttggcaggacagagatgtgtacctgcaaggacccatttgggccaaaattcctcacacggacggcaactttcacccttctccgctgatgggagggtttggaatgaaacacccgcctcctcagatcctcatcaaaaacacacctgtacctgcggatcctccaacggccttcaacaaggacaagctgaactctttcatcacccagtattctactggccaagtcagcgtggagatcgagtgggagctgcagaaggaaaacagcaagcgctggaacccggagatccagtacacttccaactattacaagtctaataatgttgaatttgctgttaatactgaaggtgtatatagtgaaccccgccccattggcaccagatacctgactcgtaatctgtaa

SEQ ID NO: 28 - protein, 744 aa, synthetic construct
  REGION 1..744: note = AAVS10_P1 capsid polypeptide
MAADGYLPDWLEDNLSEGIREWWALKPGAPKPKANQQKQDDGRGLVLPGYKYLGPFNGLDKGEPVNAADAAALEHDKAYDQQLQAGDNPYLRYNHADAEFQERLQEDTSFGGNLGRAVFQAKKRLLEPLGLVEEAAKTAPGKKRPVEQSPQEPDSSAGIGKSGAQPAKKRLNFGQTGDTESVPDPQPIGEPPAAPSGVGSLTMASGGGAPVADNNEGADGVGNASGNWHCDSQWLGDRVITTSTRTWALPTYNNHLYKQISSASTGATNDNTYFGYSTPWGYFDFNRFHCHFSPRDWQRLINNNWGFRPKRLNFKLFNIQVKEVTDNNGVKTIANNLTSTVQVFTDSDYQLPYVLGSAHEGCLPPFPADVFMIPQYGYLTLNDGSQAVGRSSFYCLEYFPSQMLRTGNNFQFSYEFENVPFHSSYAHSQSLDRLMNPLIDQYLYYLSKTINGSGQNQQTLKFSVAGPSNMAVQGRNYIPGPSYRQQRVSTTVTQNNNSEFAWPGASSWALNGRNSLMNPGPAMASHKEGEDRFFPLSGSLIFGKQGTGRDNVDADKVMITNEEEIKTTNPVATESYGQVATNHQGQSGRGDLGLSAQAAQTGWVQNQGILPGMVWQDRDVYLQGPIWAKIPHTDGNFHPSPLMGGFGMKHPPPQILIKNTPVPADPPTAFNKDKLNSFITQYSTGQVSVEIEWELQKENSKRWNPEIQYTSNYYKSNNVEFAVNTEGVYSEPRPIGTRYLTRNL

SEQ ID NO: 29 - DNA, 2235 bp, synthetic construct
  misc_feature 1..2235: note = AAVS10_P1 capsid polypeptide encoding
  source 1..2235: mol_type = other DNA
atggctgccgatggttatcttccagattggctcgaggacaacctctctgagggcattcgcgagtggtgggctttgaaacctggagccccgaagcccaaagccaaccagcaaaagcaggacgacggccggggtctggtgcttcctggctacaagtacctcggacccttcaacggactcgacaagggggagcccgtcaacgcggcggacgcagcggccctcgagcacgacaaggcctacgaccagcagctgcaggcgggtgacaatccgtacctgcggtataaccacgccgacgccgagtttcaggagcgtctgcaagaagatacgtcttttgggggcaacctcgggcgagcagtcttccaggccaaaaagaggcttcttgaacctcttggtctggttgaggaagcggctaagacggctcctggaaagaaacgtccggtagagcagtcgccacaagagccagactcctccgcgggtattggcaaatcgggtgcacagcccgctaaaaagagactcaatttcggtcagactggcgacacagagtcagtcccagaccctcaaccaatcggagaacctcccgcagccccctcaggtgtgggatctcttacaatggcttcaggtggtggcgcaccagtggcagacaataacgaaggcgccgacggagtgggtaatgcctcgggaaattggcattgcgattcccaatggctgggggacagagtcatcaccaccagcacccgaacctgggccctgcccacctacaacaatcacctctacaagcaaatctccagtgcttcaacgggggccaccaacgacaacacctacttcggctacagcaccccctgggggtattttgacttcaacagattccactgccacttctcaccacgtgactggcagcgactcatcaacaacaactggggattccggcctaagcgactcaacttcaagctcttcaacattcaggtcaaagaggttacggacaacaatggagtcaagaccatcgccaataaccttaccagcacggtccaggtcttcacggactcagactatcagctcccgtacgtgctcgggtcggctcacgagggctgcctcccgccgttcccagcggacgttttcatgattcctcagtacgggtatctgacgcttaatgatggaagccaggccgtgggtcgttcgtccttttactgcctggaatatttcccgtcgcaaatgctaagaacgggtaacaacttccagttcagctacgagtttgagaacgtacctttccatagcagctacgctcacagccaaagcctggaccgactaatgaatccactcatcgaccaatacttgtactatctctcaaagactattaacggttctggacagaatcaacaaacgctaaaattcagtgtggccggacccagcaacatggctgtccagggaagaaactacatacctggacccagctaccgacaacaacgtgtctcaaccactgtgactcaaaacaacaacagcgaatttgcttggcctggagcttcttcttgggctctcaatggacgtaatagcttgatgaatcctggacctgctatggccagccacaaagaaggagaggaccgtttctttcctttgtctggatctttaatttttggcaaacaaggaactggaagagacaacgtggatgcggacaaagtcatgataaccaacgaagaagaaattaaaactactaacccggtagcaacggagtcctatggacaagtggccacaaaccaccagggccagagtggccgcggcgatctgggcctgagcgcccaggcggcccagaccggctgggttcaaaaccaaggaatacttccgggtatggtttggcaggacagagatgtgtacctgcaaggacccatttgggccaaaattcctcacacggacggcaactttcacccttctccgctgatgggagggtttggaatgaaacacccgcctcctcagatcctcatcaaaaacacacctgtacctgcggatcctccaacggccttcaacaaggacaagctgaactctttcatcacccagtattctactggccaagtcagcgtggagatcgagtgggagctgcagaaggaaaacagcaagcgctggaacccggagatccagtacacttccaactattacaagtctaataatgttgaatttgctgttaatactgaaggtgtatatagtgaaccccgccccattggcaccagatacctgactcgtaatctgtaa

SEQ ID NO: 30 - protein, 746 aa, synthetic construct
  REGION 1..746: note = AAVS1_P1 capsid polypeptide
MAADGYLPDWLEDNLSEGIREWWALKPGAPQPKANQQHQDNARGLVLPGYKYLGPGNGLDKGEPVNAADAAALEHDKAYDQQLKAGDNPYLRYNHADAEFQERLQEDTSFGGNLGRAVFQAKKRVLEPLGLVEEGAKTAPGKKRPVEPSPQRSPDSSTGIGKTGQQPAKKRLNFGQTGDTESVPDPQPIGEPPAAPAAVGPTTMASGGGAPMADNNEGADGVGNASGNWHCDSTWLGDRVITTSTRTWALPTYNNHLYKQISNGTSGGATNDNTYFGYSTPWGYFDFNRFHCHFSPRDWQRLINNNWGFRPKRLNFKLFNIQVKEVTDNNGVKTIANNLTSTVQVFTDSDYQLPYVLGSAHEGCLPPFPADVFMIPQYGYLTLNDGSQAVGRSSFYCLEYFPSQMLRTGNNFQFSYEFENVPFHSSYAHSQSLDRLMNPLIDQYLYYLSKTINGSGQNQQTLKFSVAGPSNMAVQGRNYIPGPSYRQQRVSTTVTQNNNSEFAWPGASSWALNGRNSLMNPGPAMASHKEGEDRFFPLSGSLIFGKQGTGRDNVDADKVMITNEEEIKTTNPVATESYGQVATNHQGQSGRGDLGLSAQAAQTGWVQNQGILPGMVWQDRDVYLQGPIWAKIPHTDGNFHPSPLMGGFGMKHPPPQILIKNTPVPADPPTAFNKDKLNSFITQYSTGQVSVEIEWELQKENSKRWNPEIQYTSNYYKSNNVEFAVNTEGVYSEPRPIGTRYLTRNL

SEQ ID NO: 31 - DNA, 2241 bp, synthetic construct
  misc_feature 1..2241: note = AAVS1_P1 capsid polypeptide encoding
  source 1..2241: mol_type = other DNA
atggctgccgatggttatcttccagattggctcgaggacaaccttagtgaaggaattcgcgagtggtgggctttgaaacctggagcccctcaacccaaggcaaatcaacaacatcaagacaacgctcgaggtcttgtgcttccgggttacaaataccttggacccggcaacggactcgacaagggggagccggtcaacgcagcagacgcggcggccctcgagcacgacaaggcctacgaccagcagctcaaagcgggtgacaatccgtacctgcggtataaccacgccgacgccgagtttcaggagcgtctgcaagaagatacgtcttttgggggcaacctcgggcgagcagtcttccaggccaagaagcgggttctcgaacctctcggtctggttgaggaaggcgctaagacggctcctggaaagaaacgtccggtagagccatcaccccagcgttctccagactcctctacgggcatcggcaagacaggccagcagcccgctaaaaagagactcaatttcggtcagactggcgacacagagtcagtcccagaccctcaaccaatcggagaacctcccgcagcccccgctgctgtgggacctactacaatggcttcaggcggtggcgcaccaatggcagacaataacgaaggcgccgacggagtgggtaatgcctcaggaaattggcattgcgattccacatggctgggcgacagagtcatcaccaccagcacccgaacctgggccctgcccacctacaacaaccacctctacaagcaaatctccaacgggacatcgggaggagccaccaacgacaacacctacttcggctacagcaccccctgggggtattttgatttcaacagattccactgccatttctcaccacgtgactggcagcgactcatcaacaacaattggggattccggcccaagagactcaacttcaagctcttcaacattcaggtcaaagaggttacggacaacaatggagtcaagaccatcgccaataaccttaccagcacggtccaggtcttcacggactcagactatcagctcccgtacgtgctcgggtcggctcacgagggctgcctcccgccgttcccagcggacgttttcatgattcctcagtacgggtatctgacgcttaatgatggaagccaggccgtgggtcgttcgtccttttactgcctggaatatttcccgtcgcaaatgctaagaacgggtaacaacttccagttcagctacgagtttgagaacgtacctttccatagcagctacgctcacagccaaagcctggaccgactaatgaatccactcatcgaccaatacttgtactatctctcaaagactattaacggttctggacagaatcaacaaacgctaaaattcagtgtggccggacccagcaacatggctgtccagggaagaaactacatacctggacccagctaccgacaacaacgtgtctcaaccactgtgactcaaaacaacaacagcgaatttgcttggcctggagcttcttcttgggctctcaatggacgtaatagcttgatgaatcctggacctgctatggccagccacaaagaaggagaggaccgtttctttcctttgtctggatctttaatttttggcaaacaaggaactggaagagacaacgtggatgcggacaaagtcatgataaccaacgaagaagaaattaaaactactaacccggtagcaacggagtcctatggacaagtggccacaaaccaccagggccagagtggccgcggcgatctgggcctgagcgcccaggcggcccagaccggctgggttcaaaaccaaggaatacttccgggtatggtttggcaggacagagatgtgtacctgcaaggacccatttgggccaaaattcctcacacggacggcaactttcacccttctccgctgatgggagggtttggaatgaaacacccgcctcctcagatcctcatcaaaaacacacctgtacctgcggatcctccaacggccttcaacaaggacaagctgaactctttcatcacccagtattctactggccaagtcagcgtggagatcgagtgggagctgcagaaggaaaacagcaagcgctggaacccggagatccagtacacttccaactattacaagtctaataatgttgaatttgctgttaatactgaaggtgtatatagtgaaccccgccccattggcaccagatacctgactcgtaatctgtaa

SEQ ID NO: 32 - protein, 745 aa, synthetic construct
  REGION 1..745: note = AAVD20_P1 capsid polypeptide
MAADGYLPDWLEDNLSEGIREWWALKPGAPQPKANQQHQDNARGLVLPGYKYLGPGNGLDKGEPVNAADAAALEHDKAYDQQLKAGDNPYLKYNHADAEFQERLKEDTSFGGNLGRAVFQTKKRVLEPFGLVEEGAKTAPGKKRPVEQSPQEPDSSSGIVKTGQQPAKKRLNFGQTGDTESVPDPQPLGEPPATPSGVGSLTMASGGGAPMADNNEGADGVGNASGNWHCDSTWLGDRVITTSTRTWALPTYNNHLYKQISNGTSGGATNDNAYFGYSTPWGYFDFNRFHCHFSPRDWQRLINNNWGFRPKRLNFKLFNIQVKEVTDNNGVKTIANNLTSTVQVFTDSDYQLPYVLGSAHEGCLPPFPADVFMIPQYGYLTLNDGSQAVGRSSFYCLEYFPSQMLRTGNNFQFSYEFENVPFHSSYAHSQSLDRLMNPLIDQYLYYLSKTINGSGQNQQTLKFSVAGPSNMAVQGRNYIPGPSYRQQRVSTTVTQNNNSEFAWPGASSWALNGRNSLMNPGPAMASHKEGEDRFFPLSGSLIFGKQGTGRDNVDADKVMITNEEEIKTTNPVATESYGQVATNHQGQSGRGDLGLSAQAAQTGWVQNQGILPGMVWQDRDVYLQGPIWAKIPHTDGNFHPSPLMGGFGMKHPPPQILIKNTPVPADPPTAFNKDKLNSFITQYSTGQVSVEIEWELQKENSKRWNPEIQYTSNYYKSNNVEFAVNTEGVYSEPRPIGTRYLTRNL

SEQ ID NO: 33 - DNA, 2238 bp, synthetic construct
  misc_feature 1..2238: note = AAVD20_P1 capsid polypeptide encoding
  source 1..2238: mol_type = other DNA
atggctgccgatggttatcttccagattggctcgaggacaaccttagtgaaggaattcgcgagtggtgggctttgaaacctggagcccctcaacccaaggcaaatcaacaacatcaagacaacgctcgaggtcttgtgcttccgggttacaaataccttggacccggcaacggactcgacaagggggagccggtcaacgcagcagacgcggcggccctcgagcacgacaaggcctacgaccagcagctcaaggccggagacaacccgtacctcaagtacaaccacgccgacgccgagttccaggagcggctcaaagaagatacgtcttttgggggcaacctcgggcgagcagtcttccagaccaagaagagggttctcgaaccttttggtctggttgaggaaggtgctaagacggctcctggaaagaaacgtccggtagagcagtcgccacaagagccagactcctcctcgggcattgtcaagacaggccagcagcccgctaaaaagagactcaattttggtcagactggcgacacagagtcagtccccgacccacaacctctcggagaacctccagcaaccccctcaggtgtgggatctcttacaatggcttcaggcggtggcgcaccaatggcagacaataacgaaggcgccgacggagtgggtaatgcctcaggaaattggcattgcgattccacatggctgggcgacagagtcatcaccaccagcacccgaacctgggccctgcccacctacaacaaccacctctacaagcaaatctccaacgggacatcgggaggagccaccaacgacaacgcctacttcggctacagcaccccctgggggtattttgactttaacagattccactgccacttttcaccacgtgactggcagcgactcatcaacaacaactggggattccggcctaagcgactcaacttcaagctcttcaacattcaggtcaaagaggttacggacaacaatggagtcaagaccatcgccaataaccttaccagcacggtccaggtcttcacggactcagactatcagctcccgtacgtgctcgggtcggctcacgagggctgcctcccgccgttcccagcggacgttttcatgattcctcagtacgggtatctgacgcttaatgatggaagccaggccgtgggtcgttcgtccttttactgcctggaatatttcccgtcgcaaatgctaagaacgggtaacaacttccagttcagctacgagtttgagaacgtacctttccatagcagctacgctcacagccaaagcctggaccgactaatgaatccactcatcgaccaatacttgtactatctctcaaagactattaacggttctggacagaatcaacaaacgctaaaattcagtgtggccggacccagcaacatggctgtccagggaagaaactacatacctggacccagctaccgacaacaacgtgtctcaaccactgtgactcaaaacaacaacagcgaatttgcttggcctggagcttcttcttgggctctcaatggacgtaatagcttgatgaatcctggacctgctatggccagccacaaagaaggagaggaccgtttctttcctttgtctggatctttaatttttggcaaacaaggaactggaagagacaacgtggatgcggacaaagtcatgataaccaacgaagaagaaattaaaactactaacccggtagcaacggagtcctatggacaagtggccacaaaccaccagggccagagtggccgcggcgatctgggcctgagcgcccaggcggcccagaccggctgggttcaaaaccaaggaatacttccgggtatggtttggcaggacagagatgtgtacctgcaaggacccatttgggccaaaattcctcacacggacggcaactttcacccttctccgctgatgggagggtttggaatgaaacacccgcctcctcagatcctcatcaaaaacacacctgtacctgcggatcctccaacggccttcaacaaggacaagctgaactctttcatcacccagtattctactggccaagtcagcgtggagatcgagtgggagctgcagaaggaaaacagcaagcgctggaacccggagatccagtacacttccaactattacaagtctaataatgttgaatttgctgttaatactgaaggtgtatatagtgaaccccgccccattggcaccagatacctgactcgtaatctgtaa

SEQ ID NO: 34 - protein, 745 aa, synthetic construct
  REGION 1..745: note = AAVH15_P1 capsid polypeptide
MAADGYLPDWLEDNLSEGIREWWDLKPGAPKPKANQQKQDDGRGLVLPGYKYLGPFNGLDKGEPVNAADAAALEHDKAYDQQLKAGDNPYLRYNHADAEFQERLQEDTSFGGNLGRAVFQAKKRVLEPFGLVEEGAKTAPGKKRPVEQSPQEPDSSSGIGKTGQQPAKKRLNFGQTGDSESVPDPQPLGEPPATPAAVGPTTMASGGGAPVADNNEGADGVGSSSGNWHCDSQWLGDRVITTSTRTWALPTYNNHLYKQISNSTSGGSSNDNAYFGYSTPWGYFDFNRFHCHFSPRDWQRLINNNWGFRPKRLNFKLFNIQVKEVTDNNGVKTIANNLTSTVQVFTDSDYQLPYVLGSAHEGCLPPFPADVFMIPQYGYLTLNDGSQAVGRSSFYCLEYFPSQMLRTGNNFQFSYEFENVPFHSSYAHSQSLDRLMNPLIDQYLYYLSKTINGSGQNQQTLKFSVAGPSNMAVQGRNYIPGPSYRQQRVSTTVTQNNNSEFAWPGASSWALNGRNSLMNPGPAMASHKEGEDRFFPLSGSLIFGKQGTGRDNVDADKVMITNEEEIKTTNPVATESYGQVATNHQGQSGRGDLGLSAQAAQTGWVQNQGILPGMVWQDRDVYLQGPIWAKIPHTDGNFHPSPLMGGFGLKHPPPQILIKNTPVPADPPAEFSATKFASFITQYSTGQVSVEIEWELQKENSKRWNPEVQYTSNYAKSANVDFTVDNNGLYTEPRPIGTRYLTRPL

SEQ ID NO: 35 - DNA, 2238 bp, synthetic construct
  misc_feature 1..2238: note = AAVH15_P1 capsid polypeptide encoding
  source 1..2238: mol_type = other DNA
atggctgccgatggttatcttccagattggctcgaggacaacctctctgagggcattcgcgagtggtgggacttgaaacctggagccccgaaacccaaagccaaccagcaaaagcaggacgacggccggggtctggtgcttcctggctacaagtacctcggacccttcaacggactcgacaagggggagcccgtcaacgcggcggatgcagcggccctcgagcacgacaaggcctacgaccagcagctcaaagcgggtgacaatccgtaccttcggtataaccacgccgacgccgagtttcaggagcgtctgcaagaagatacgtcttttgggggcaacctcgggcgagcagtcttccaggccaagaagagggttctcgaaccttttggtctggttgaggaaggtgctaagacggctcctggaaagaaacgtccggtagagcagtcgccacaagagccagactcctcctcgggcattggcaagacaggccagcagcccgctaaaaagagactcaattttggtcagactggcgactcagagtcagtccccgacccacaacctctcggagaacctccagcaacccccgctgctgtgggacctactacaatggcttcaggtggtggcgcaccagtggcagacaataacgaaggtgccgatggagtgggtagttcctcgggaaattggcattgcgattcccaatggctgggggacagagtcatcaccaccagcacccgaacctgggccctgcccacctacaacaatcacctctacaagcaaatctccaacagcacatctggaggatcttcaaatgacaacgcctacttcggctacagcaccccctgggggtattttgacttcaacagattccactgccacttctcaccacgtgactggcagcgactcatcaacaacaactggggattccggcctaagcgactcaacttcaagctcttcaacattcaggtcaaagaggttacggacaacaatggagtcaagaccatcgccaataaccttaccagcacggtccaggtcttcacggactcagactatcagctcccgtacgtgctcgggtcggctcacgagggctgcctcccgccgttcccagcggacgttttcatgattcctcagtacgggtatctgacgcttaatgatggaagccaggccgtgggtcgttcgtccttttactgcctggaatatttcccgtcgcaaatgctaagaacgggtaacaacttccagttcagctacgagtttgagaacgtacctttccatagcagctacgctcacagccaaagcctggaccgactaatgaatccactcatcgaccaatacttgtactatctctcaaagactattaacggttctggacagaatcaacaaacgctaaaattcagtgtggccggacccagcaacatggctgtccagggaagaaactacatacctggacccagctaccgacaacaacgtgtctcaaccactgtgactcaaaacaacaacagcgaatttgcttggcctggagcttcttcttgggctctcaatggacgtaatagcttgatgaatcctggacctgctatggccagccacaaagaaggagaggaccgtttctttcctttgtctggatctttaatttttggcaaacaaggaactggaagagacaacgtggatgcggacaaagtcatgataaccaacgaagaagaaattaaaactactaacccggtagcaacggagtcctatggacaagtggccacaaaccaccagggccagagtggccgcggcgatctgggcctgagcgcccaggcggcccagaccggctgggttcaaaaccaaggaatacttccgggtatggtttggcaggacagagatgtgtacctgcaaggacccatttgggccaaaattcctcacacggacggcaacttccacccgtctccgctgatgggcggctttggcctgaaacatcctccgcctcagatcctgatcaagaacacgcctgtacctgcggatcctccggcagagttttcggctacaaagtttgcttcattcatcacccagtattccacaggacaagtgagcgtggagattgaatgggagctgcagaaagaaaacagcaaacgctggaatcccgaagtgcagtatacatctaactatgcaaaatctgccaacgttgatttcactgtggacaacaatggactttatactgagcctcgccccattggcacccgttacctcacccgtcccctgtaa

SEQ ID NO: 36 - protein, 6 aa, synthetic construct
  REGION 1..6: note = AAV1 insertion site 1
STDPAT

SEQ ID NO: 37 - protein, 6 aa, synthetic construct
  REGION 1..6: note = AAV1 insertion site 2
SSSTDP

SEQ ID NO: 38 - protein, 6 aa, synthetic construct
  REGION 1..6: note = AAV2 insertion site 1
GNRQAA

SEQ ID NO: 39 - protein, 6 aa, synthetic construct
  REGION 1..6: note = AAV2 insertion site 2
RGNRQA

SEQ ID NO: 40 - protein, 6 aa, synthetic construct
  REGION 1..6: note = AAV3b insertion site 1
LQSSNT

SEQ ID NO: 41 - protein, 6 aa, synthetic construct
  REGION 1..6: note = AAV3b insertion site 2
SSNTAP

SEQ ID NO: 42 - protein, 6 aa, synthetic construct
  REGION 1..6: note = AAV4 insertion site 1
DQSNSN

SEQ ID NO: 43 - protein, 6 aa, synthetic construct
  REGION 1..6: note = AAV4 insertion site 2
SNSNLP

SEQ ID NO: 44 - protein, 6 aa, synthetic construct
  REGION 1..6: note = AAV5 insertion site 1
NQSSTT

SEQ ID NO: 45 - protein, 6 aa, synthetic construct
  REGION 1..6: note = AAV5 insertion site 2
SSTTAP

SEQ ID NO: 46 - protein, 6 aa, synthetic construct
  REGION 1..6: note = AAV6 insertion site 1
STDPAT

SEQ ID NO: 47 - protein, 6 aa, synthetic construct
  REGION 1..6: note = AAV6 insertion site 2
SSSTDP

SEQ ID NO: 48 - protein, 6 aa, synthetic construct
  REGION 1..6: note = AAV7 insertion site 1
AANTAA

SEQ ID NO: 49 - protein, 6 aa, synthetic construct
  REGION 1..6: note = AAV8 insertion site 1
QQNTAP

SEQ ID NO: 50 - protein, 6 aa, synthetic construct
  REGION 1..6: note = AAV9 insertion site 1
SAQAQA

SEQ ID NO: 51 - protein, 6 aa, synthetic construct
  REGION 1..6: note = AAVrh10 insertion site 1
QQNAAP

SEQ ID NO: 52 - protein, 6 aa, synthetic construct
  REGION 1..6: note = AAVpo.1 insertion site 1
NQNSNT

SEQ ID NO: 53 - protein, 6 aa, synthetic construct
  REGION 1..6: note = AAVpo.1 insertion site 2
NSNTHP

SEQ ID NO: 54 - protein, 6 aa, synthetic construct
  REGION 1..6: note = AAV12 insertion site 1
NQNATT

SEQ ID NO: 55 - protein, 6 aa, synthetic construct
  REGION 1..6: note = AAV12 insertion site 2
NATTAP